European Patent Application EP 4 299 747 A1, published January 3, 2024. Title: MAD7 mutant protein. Applicant: 株式会社セツロテック. Application JP. The sequence listing filed with the application follows.

SEQUENCE LISTING (10 sequences)

SEQ ID NO: 1 - protein, 1263 aa, synthetic construct
  source 1..1263: note = MAD7
MNNGTNNFQNFIGISSLQKTLRNALIPTETTQQFIVKNGIIKEDELRGENRQILKDIMDDYYRGFISETLSSIDDIDWTSLFEKMEIQLKNGDNKDTLIKEQTEYRKAIHKKFANDDRFKNMFSAKLISDILPEFVIHNNNYSASEKEEKTQVIKLFSRFATSFKDYFKNRANCFSADDISSSSCHRIVNDNAEIFFSNALVYRRIVKSLSNDDINKISGDMKDSLKEMSLEEIYSYEKYGEFITQEGISFYNDICGKVNSFMNLYCQKNKENKNLYKLQKLHKQILCIADTSYEVPYKFESDEEVYQSVNGFLDNISSKHIVERLRKIGDNYNGYNLDKIYIVSKFYESVSQKTYRDWETINTALEIHYNNILPGNGKSKADKVKKAVKNDLQKSITEINELVSNYKLCSDDNIKAETYIHEISHILNNFEAQELKYNPEIHLVESELKASELKNVLDVIMNAFHWCSVFMTEELVDKDNNFYAELEEIYDEIYPVISLYNLVRNYVTQKPYSTKKIKLNFGIPTLADGWSKSKEYSNNAIILMRDNLYYLGIFNAKNKPDKKIIEGNTSENKGDYKKMIYNLLPGPNKMIPKVFLSSKTGVETYKPSAYILEGYKQNKHIKSSKDFDITFCHDLIDYFKNCIAIHPEWKNFGFDFSDTSTYEDISGFYREVELQGYKIDWTYISEKDIDLLQEKGQLYLFQIYNKDFSKKSTGNDNLHTMYLKNLFSEENLKDIVLKLNGEAEIFFRKSSIKNPIIHKKGSILVNRTYEAEEKDQFGNIQIVRKNIPENIYQELYKYFNDKSDKELSDEAAKLKNVVGHHEAATNIVKDYRYTYDKYFLHMPITINFKANKTGFINDRILQYIAKEKDLHVIGIDRGERNLIYVSVIDTCGNIVEQKSFNIVNGYDYQIKLKQQEGARQIARKEWKEIGKIKEIKEGYLSLVIHEISKMVIKYNAIIAMEDLSYGFKKGRFKVERQVYQKFETMLINKLNYLVFKDISITENGGLLKGYQLTYIPDKLKNVGHQCGCIFYVPAAYTSKIDPTTGFVNIFKFKDLTVDAKREFIKKFDSIRYDSEKNLFCFTFDYNNFITQNTVMSKSSWSVYTYGVRIKRRFVNGRFSNESDTIDITKDMEKTLEMTDINWRDGHDLRQDIIDYEIVQHIFEIFRLTVQMRNSLSELEDRDYDRLISPVLNENNIFYDSAKAGDALPKDADANGAYCIALKGLYEIKQITENWKEDGKFSRDKLKISNKDWFDFIQNKRYL

SEQ ID NO: 2 - protein, 1263 aa, synthetic construct
  source 1..1263: note = ST8-1s
MNNGTNNFQNFIGISSLQKTLRNALIPTETTQQFIVKNGIIKEDELRGENRQILKDIMDDYYRGFISETLSSIDDIDWTSLFEKMEIQLKNGDNKDTLIKEQTEYRKAIHKKFANDDRFKNMFSAKLISDILPEFVIHNNNYSASEKEEKTQVIKLFSRFATSFKDYFRNRANCFSADDISSSSCHRIVNDNAEIFFSNALVYRRIVKSLSNDDINKISGDMKDSLKEMSLEEIYSYEKYGEFITQEGISFYNDICGKVNSFMNLYCQKNKENKNLYKLQKLHKQILCIADTSYEVPYKFESDEEVYQSVNGFLDNISSKHIVERLRKIGDNYNGYNLDKIYIVSKFYESVSQKTYRDWETINTALEIHYNNILPGNGKSKADKVKKAVKNDLQKSITEINELVSNYKLCSDDNIKAETYIHEISHILNNFEAQELKYNPEIHLVESELKASELKNVLDVIMNAFHWCSVFMTEELVDKDNNFYAELEEIYDEIYPVISLYNLVRNYVTQKPYSTKKIKLNFGIPTLARGWSKSKEYSNNAIILMRDNLYYLGIFNAKNKPDKKIIEGNTSENKGDYKKMIYNLLPGPNKMIPKVFLSSKTGVETYKPSAYILEGYKQNKHIKSSKDFDITFCHDLIDYFKNCIAIHPEWKNFGFDFSDTSTYEDISGFYREVELQGYKIDWTYISEKDIDLLQEKGQLYLFQIYNKDFSKKSTGNDNLHTMYLKNLFSEENLKDIVLKLNGEAEIFFRKSSIKNPIIHKKGSILVNRTYEAEEKDQFGNIQIVRKNIPENIYQELYKYFNDKSDKELSDEAAKLKNVVGHHEAATNIVKDYRYTYDKYFLHMPITINFKANKTGFINDRILQYIAKEKDLHVIGIDRGERNLIYVSVIDTCGNIVEQKSFNIVNGYDYQIKLKQQEGARQIARKEWKEIGKIKEIKEGYLSLVIHEISKMVIKYNAIIAMEDLSYGFKNGRFKVERQVYQKFETMLINKLNYLVFKDISITENGGLLKGYQLTYIPDKLKNVGHQCGCIFYVPAAYTSKIDPTTGFVNIFKFKDLTVDAKREFIKKFDSIRYDSEKNLFCFTFDFNNFITQNTVMSKSSWSVYTYGVRIKRRFVNGRFSNESDTIDITKDMEKTLEMTDINWRDGHDLRQDIIDYEIVQHIFEIFRLTVQMRNSLSELEDRDYDRLISPVLNENNIFYDSAKAGDALPKDADANGAYCIALKGLYEIKQITENWKEDGKFSRDKLKISNKDWFDFIQNKRYL

SEQ ID NO: 3 - protein, 1263 aa, synthetic construct
  source 1..1263: note = ST8-2s
MNNGTNNFQNFIGISSLQKTLRNALIPTETTQQFIVKNGIIKEDELRGENRQILKDIMDDYYRGFISETLSSIDDIDWTSLFEKMEIQLKNGDNKDTLIKEQTEYRKAIHKKFANDDRFKNMFSAKLISDILPEFVIHNNNYSASEKEEKTQVIKLFSRFATSFKDYFRNRANCFSADDISSSSCHRIVNDNAEIFFSNALVYRRIVKSLSNDDINKISGDMKDSLKEMSLEEIYSYEKYGEFITQEGISFYNDICGKVNSFMNLYCQKNKENKNLYKLQKLHKQILCIADTSYEVPYKFESDEEVYQSVNGFLDNISSKHIVERLRKIGDNYNGYNLDKIYIVSKFYESVSQKTYRDWETINTALEIHYNNILPGNGKSKADKVKKAVKNDLQKSITEINELVSNYKLCSDDNIKAETYIHEISHILNNFEAQELKYNPEIHLVESELKASELKNVLDVIMNAFHWCSVFMTEELVDKDNNFYAELEEIYDEIYPVISLYNLVRNYVTQKPYSTKKIKLNFGIPTLARGWSKSKEYSNNAIILMRDNLYYLGIFNAKNKPDKKIIEGNTSENKGDYKKMIYNLLPGPNKMIPKVFLSSKTGVETYKPSAYILEGYKQNKHIKSSKDFDITFCHDLIDYFKNCIAIHPEWKNFGFDFSDTSTYEDISGFYREVELQGYKIDWTYISEKDIDLLQEKGQLYLFQIYNKDFSKKSTGNDNLHTMYLKNLFSEENLKDIVLKLNGEAEIFFRKSSIKNPIIHKKGSILVNRTYEAEEKDQFGNIQIVRKNIPENIYQELYKYFNDKSDKELSDEAAKLKNVVGHHEAATNIVKDYRYTYDKYFLHMPITINFKANKTGFINDRILQYIAKEKDLHVIGIDRGERNLIYVSVIDTCGNIVEQKSFNIVNGYDYQIKLKQQEGARQIARKEWKEIGKIKEIKEGYLSLVIHEISKMVIKYNAIIAMEDLSYGFKKGRFKVERQVYQKFETMLINKLNYLVFKDISITENGGLLKGYQLTYIPDKLKNVGHQCGCIFYVPAAYTSKIDPTTGFVNIFKFKDLTVDAKREFIKKFDSIRYDSEKNLFCFTFDFNNFITQNTVMSKSSWSVYTYGVRIKRRFVNGRFSNESDTIDITKDMEKTLEMTDINWRDGHDLRQDIIDYEIVQHIFEIFRLTVQMRNSLSELEDRDYDRLISPVLNENNIFYDSAKAGDALPKDADANGAYCIALKGLYKIKQITENWKEDGKFSRDKLKISNKDWFDFIQNKRYL

SEQ ID NO: 4 - protein, 16 aa, synthetic construct
  source 1..16: note = NLS
KRPAATKKAGQAKKKK

SEQ ID NO: 5 - protein, 27 aa, synthetic construct
  source 1..27: note = 3xHA
YPYDVPDYAYPYDVPDYAYPYDVPDYA

SEQ ID NO: 6 - RNA, 41 nt, synthetic construct
  source 1..41: mol_type = other RNA; note = crRNA-1
taatttctactcttgtagattgtcaccaatcctgtccctag

SEQ ID NO: 7 - RNA, 41 nt, synthetic construct
  source 1..41: mol_type = other RNA; note = crRNA-2
taatttctactcttgtagatcacctgttcaattcccctgca

SEQ ID NO: 8 - protein, 1308 aa, synthetic construct
  source 1..1308: note = ST7
MNNGTNNFQNFIGISSLQKTLRNALIPTETTQQFIVKNGIIKEDELRGENRQILKDIMDDYYRGFISETLSSIDDIDWTSLFEKMEIQLKNGDNKDTLIKEQTEYRKAIHKKFANDDRFKNMFSAKLISDILPEFVIHNNNYSASEKEEKTQVIKLFSRFATSFKDYFKNRANCFSADDISSSSCHRIVNDNAEIFFSNALVYRRIVKSLSNDDINKISGDMKDSLKEMSLEEIYSYEKYGEFITQEGISFYNDICGKVNSFMNLYCQKNKENKNLYKLQKLHKQILCIADTSYEVPYKFESDEEVYQSVNGFLDNISSKHIVERLRKIGDNYNGYNLDKIYIVSKFYESVSQKTYRDWETINTALEIHYNNILPGNGKSKADKVKKAVKNDLQKSITEINELVSNYKLCSDDNIKAETYIHEISHILNNFEAQELKYNPEIHLVESELKASELKNVLDVIMNAFHWCSVFMTEELVDKDNNFYAELEEIYDEIYPVISLYNLVRNYVTQKPYSTKKIKLNFGIPTLADGWSKSKEYSNNAIILMRDNLYYLGIFNAKNKPDKKIIEGNTSENKGDYKKMIYNLLPGPNKMIPKVFLSSKTGVETYKPSAYILEGYKQNKHIKSSKDFDITFCHDLIDYFKNCIAIHPEWKNFGFDFSDTSTYEDISGFYREVELQGYKIDWTYISEKDIDLLQEKGQLYLFQIYNKDFSKKSTGNDNLHTMYLKNLFSEENLKDIVLKLNGEAEIFFRKSSIKNPIIHKKGSILVNRTYEAEEKDQFGNIQIVRKNIPENIYQELYKYFNDKSDKELSDEAAKLKNVVGHHEAATNIVKDYRYTYDKYFLHMPITINFKANKTGFINDRILQYIAKEKDLHVIGIDRGERNLIYVSVIDTCGNIVEQKSFNIVNGYDYQIKLKQQEGARQIARKEWKEIGKIKEIKEGYLSLVIHEISKMVIKYNAIIAMEDLSYGFKKGRFKVERQVYQKFETMLINKLNYLVFKDISITENGGLLKGYQLTYIPDKLKNVGHQCGCIFYVPAAYTSKIDPTTGFVNIFKFKDLTVDAKREFIKKFDSIRYDSEKNLFCFTFDYNNFITQNTVMSKSSWSVYTYGVRIKRRFVNGRFSNESDTIDITKDMEKTLEMTDINWRDGHDLRQDIIDYEIVQHIFEIFRLTVQMRNSLSELEDRDYDRLISPVLNENNIFYDSAKAGDALPKDADANGAYCIALKGLYEIKQITENWKEDGKFSRDKLKISNKDWFDFIQNKRYLKRPAATKKAGQAKKKKGSYPYDVPDYAYPYDVPDYAYPYDVPDYA

SEQ ID NO: 9 - protein, 1308 aa, synthetic construct
  source 1..1308: note = ST8-1
MNNGTNNFQNFIGISSLQKTLRNALIPTETTQQFIVKNGIIKEDELRGENRQILKDIMDDYYRGFISETLSSIDDIDWTSLFEKMEIQLKNGDNKDTLIKEQTEYRKAIHKKFANDDRFKNMFSAKLISDILPEFVIHNNNYSASEKEEKTQVIKLFSRFATSFKDYFRNRANCFSADDISSSSCHRIVNDNAEIFFSNALVYRRIVKSLSNDDINKISGDMKDSLKEMSLEEIYSYEKYGEFITQEGISFYNDICGKVNSFMNLYCQKNKENKNLYKLQKLHKQILCIADTSYEVPYKFESDEEVYQSVNGFLDNISSKHIVERLRKIGDNYNGYNLDKIYIVSKFYESVSQKTYRDWETINTALEIHYNNILPGNGKSKADKVKKAVKNDLQKSITEINELVSNYKLCSDDNIKAETYIHEISHILNNFEAQELKYNPEIHLVESELKASELKNVLDVIMNAFHWCSVFMTEELVDKDNNFYAELEEIYDEIYPVISLYNLVRNYVTQKPYSTKKIKLNFGIPTLARGWSKSKEYSNNAIILMRDNLYYLGIFNAKNKPDKKIIEGNTSENKGDYKKMIYNLLPGPNKMIPKVFLSSKTGVETYKPSAYILEGYKQNKHIKSSKDFDITFCHDLIDYFKNCIAIHPEWKNFGFDFSDTSTYEDISGFYREVELQGYKIDWTYISEKDIDLLQEKGQLYLFQIYNKDFSKKSTGNDNLHTMYLKNLFSEENLKDIVLKLNGEAEIFFRKSSIKNPIIHKKGSILVNRTYEAEEKDQFGNIQIVRKNIPENIYQELYKYFNDKSDKELSDEAAKLKNVVGHHEAATNIVKDYRYTYDKYFLHMPITINFKANKTGFINDRILQYIAKEKDLHVIGIDRGERNLIYVSVIDTCGNIVEQKSFNIVNGYDYQIKLKQQEGARQIARKEWKEIGKIKEIKEGYLSLVIHEISKMVIKYNAIIAMEDLSYGFKNGRFKVERQVYQKFETMLINKLNYLVFKDISITENGGLLKGYQLTYIPDKLKNVGHQCGCIFYVPAAYTSKIDPTTGFVNIFKFKDLTVDAKREFIKKFDSIRYDSEKNLFCFTFDFNNFITQNTVMSKSSWSVYTYGVRIKRRFVNGRFSNESDTIDITKDMEKTLEMTDINWRDGHDLRQDIIDYEIVQHIFEIFRLTVQMRNSLSELEDRDYDRLISPVLNENNIFYDSAKAGDALPKDADANGAYCIALKGLYEIKQITENWKEDGKFSRDKLKISNKDWFDFIQNKRYLKRPAATKKAGQAKKKKGSYPYDVPDYAYPYDVPDYAYPYDVPDYA

SEQ ID NO: 10 - protein, 1308 aa, synthetic construct
  source 1..1308: note = ST8-2
MNNGTNNFQNFIGISSLQKTLRNALIPTETTQQFIVKNGIIKEDELRGENRQILKDIMDDYYRGFISETLSSIDDIDWTSLFEKMEIQLKNGDNKDTLIKEQTEYRKAIHKKFANDDRFKNMFSAKLISDILPEFVIHNNNYSASEKEEKTQVIKLFSRFATSFKDYFRNRANCFSADDISSSSCHRIVNDNAEIFFSNALVYRRIVKSLSNDDINKISGDMKDSLKEMSLEEIYSYEKYGEFITQEGISFYNDICGKVNSFMNLYCQKNKENKNLYKLQKLHKQILCIADTSYEVPYKFESDEEVYQSVNGFLDNISSKHIVERLRKIGDNYNGYNLDKIYIVSKFYESVSQKTYRDWETINTALEIHYNNILPGNGKSKADKVKKAVKNDLQKSITEINELVSNYKLCSDDNIKAETYIHEISHILNNFEAQELKYNPEIHLVESELKASELKNVLDVIMNAFHWCSVFMTEELVDKDNNFYAELEEIYDEIYPVISLYNLVRNYVTQKPYSTKKIKLNFGIPTLARGWSKSKEYSNNAIILMRDNLYYLGIFNAKNKPDKKIIEGNTSENKGDYKKMIYNLLPGPNKMIPKVFLSSKTGVETYKPSAYILEGYKQNKHIKSSKDFDITFCHDLIDYFKNCIAIHPEWKNFGFDFSDTSTYEDISGFYREVELQGYKIDWTYISEKDIDLLQEKGQLYLFQIYNKDFSKKSTGNDNLHTMYLKNLFSEENLKDIVLKLNGEAEIFFRKSSIKNPIIHKKGSILVNRTYEAEEKDQFGNIQIVRKNIPENIYQELYKYFNDKSDKELSDEAAKLKNVVGHHEAATNIVKDYRYTYDKYFLHMPITINFKANKTGFINDRILQYIAKEKDLHVIGIDRGERNLIYVSVIDTCGNIVEQKSFNIVNGYDYQIKLKQQEGARQIARKEWKEIGKIKEIKEGYLSLVIHEISKMVIKYNAIIAMEDLSYGFKKGRFKVERQVYQKFETMLINKLNYLVFKDISITENGGLLKGYQLTYIPDKLKNVGHQCGCIFYVPAAYTSKIDPTTGFVNIFKFKDLTVDAKREFIKKFDSIRYDSEKNLFCFTFDFNNFITQNTVMSKSSWSVYTYGVRIKRRFVNGRFSNESDTIDITKDMEKTLEMTDINWRDGHDLRQDIIDYEIVQHIFEIFRLTVQMRNSLSELEDRDYDRLISPVLNENNIFYDSAKAGDALPKDADANGAYCIALKGLYKIKQITENWKEDGKFSRDKLKISNKDWFDFIQNKRYLKRPAATKKAGQAKKKKGSYPYDVPDYAYPYDVPDYAYPYDVPDYA